European Patent Application EP 4 431 606 A1, published September 18, 2024. Title: Anti-EphA4 antibody. Applicant: EISAI R&D MANAGEMENT CO., LTD. The sequence listing filed with the application follows.

SEQUENCE LISTING (126 sequences)

SEQ ID NO: 1 - protein, 986 aa, Homo sapiens
MAGIFYFALFSCLFGICDAVTGSRVYPANEVTLLDSRSVQGELGWIASPLEGGWEEVSIMDEKNTPIRTYQVCNVMEPSQNNWLRTDWITREGAQRVYIEIKFTLRDCNSLPGVMGTCKETFNLYYYESDNDKERFIRENQFVKIDTIAADESFTQVDIGDRIMKLNTEIRDVGPLSKKGFYLAFQDVGACIALVSVRVFYKKCPLTVRNLAQFPDTITGADTSSLVEVRGSCVNNSEEKDVPKMYCGADGEWLVPIGNCLCNAGHEERSGECQACKIGYYKALSTDATCAKCPPHSYSVWEGATSCTCDRGFFRADNDAASMPCTRPPSAPLNLISNVNETSVNLEWSSPQNTGGRQDISYNVVCKKCGAGDPSKCRPCGSGVHYTPQQNGLKTTKVSITDLLAHTNYTFEIWAVNGVSKYNPNPDQSVSVTVTTNQAAPSSIALVQAKEVTRYSVALAWLEPDRPNGVILEYEVKYYEKDQNERSYRIVRTAARNTDIKGLNPLTSYVFHVRARTAAGYGDFSEPLEVTTNTVPSRIIGDGANSTVLLVSVSGSVVLVVILIAAFVISRRRSKYSKAKQEADEEKHLNQGVRTYVDPFTYEDPNQAVREFAKEIDASCIKIEKVIGVGEFGEVCSGRLKVPGKREICVAIKTLKAGYTDKQRRDFLSEASIMGQFDHPNIIHLEGVVTKCKPVMIITEYMENGSLDAFLRKNDGRFTVIQLVGMLRGIGSGMKYLSDMSYVHRDLAARNILVNSNLVCKVSDFGMSRVLEDDPEAAYTTRGGKIPIRWTAPEAIAYRKFTSASDVWSYGIVMWEVMSYGERPYWDMSNQDVIKAIEEGYRLPPPMDCPIALHQLMLDCWQKERSDRPKFGQIVNMLDKLIRNPNSLKRTGTESSRPNTALLDPSSPEFSAVVSVGDWLQAIKMDRYKDNFTAAGYTTLEAVVHVNQEDLARIGITAITHQNKILSSVQAMRTQMQQMHGRMVPV

SEQ ID NO: 2 - protein, 528 aa, Homo sapiens
VTGSRVYPANEVTLLDSRSVQGELGWIASPLEGGWEEVSIMDEKNTPIRTYQVCNVMEPSQNNWLRTDWITREGAQRVYIEIKFTLRDCNSLPGVMGTCKETFNLYYYESDNDKERFIRENQFVKIDTIAADESFTQVDIGDRIMKLNTEIRDVGPLSKKGFYLAFQDVGACIALVSVRVFYKKCPLTVRNLAQFPDTITGADTSSLVEVRGSCVNNSEEKDVPKMYCGADGEWLVPIGNCLCNAGHEERSGECQACKIGYYKALSTDATCAKCPPHSYSVWEGATSCTCDRGFFRADNDAASMPCTRPPSAPLNLISNVNETSVNLEWSSPQNTGGRQDISYNVVCKKCGAGDPSKCRPCGSGVHYTPQQNGLKTTKVSITDLLAHTNYTFEIWAVNGVSKYNPNPDQSVSVTVTTNQAAPSSIALVQAKEVTRYSVALAWLEPDRPNGVILEYEVKYYEKDQNERSYRIVRTAARNTDIKGLNPLTSYVFHVRARTAAGYGDFSEPLEVTTNTVPSRIIGDGANST

SEQ ID NO: 3 - protein, 1030 aa, synthetic construct
  REGION 1..1030: note = Synthetic polypeptide
VTGSRVYPANEVTLLDSRSVQGELGWIASPLEGGWEEVSIMDEKNTPIRTYQVCNVMEPSQNNWLRTDWITREGAQRVYIEIKFTLRDCNSLPGVMGTCKETFNLYYYESDNDKERFIRENQFVKIDTIAADESFTQVDIGDRIMKLNTEIRDVGPLSKKGFYLAFQDVGACIALVSVRVFYKKCPLTVRNLAQFPDTITGADTSSLVEVRGSCVNNSEEKDVPKMYCGADGEWLVPIGNCLCNAGHEERSGECQACKIGYYKALSTDATCAKCPPHSYSVWEGATSCTCDRGFFRADNDAASMPCTRPPSAPLNLISNVNETSVNLEWSSPQNTGGRQDISYNVVCKKCGAGDPSKCRPCGSGVHYTPQQNGLKTTKVSITDLLAHTNYTFEIWAVNGVSKYNPNPDQSVSVTVTTNQAAPSSIALVQAKEVTRYSVALAWLEPDRPNGVILEYEVKYYEKDQNERSYRIVRTAARNTDIKGLNPLTSYVFHVRARTAAGYGDFSEPLEVTTNTVPSRIIGDGANSTAAAIIPVEEENPDFWNREAAEALGAAKKLQPAQTAAKNLIIFLGDGMGVSTVTAARILKGQKKDKLGPEIPLAMDRFPYVALSKTYNVDKHVPDSGATATAYLCGVKGNFQTIGLSAAARFNQCNTTRGNEVISVMNRAKKAGKSVGVVTTTRVQHASPAGTYAHTVNRNWYSDADVPASARQEGCQDIATQLISNMDIDVILGGGRKYMFRMGTPDPEYPDDYSQGGTRLDGKNLVQEWLAKRQGARYVWNRTELMQASLDPSVTHLMGLFEPGDMKYEIHRDSTLDPSLMEMTEAALRLLSRNPRGFFLFVEGGRIDHGHHESRAYRALTETIMFDDAIERAGQLTSEEDTLSLVTADHSHVFSFGGYPLRGSSIFGLAPGKARDRKAYTVLLYGNGPGYVLKDGARPDVTESESGSPEYRQQSAVPLDEETHAGEDVAVFARGPQAHLVHGVQEQTFIAHVMAFAACLEPYTACDLAPPAGTTDAAHPGHHHHHHHHHH

SEQ ID NO: 4 - protein, 541 aa, synthetic construct
  REGION 1..541: note = Synthetic polypeptide
VTGSRVYPANEVTLLDSRSVQGELGWIASPLEGGWEEVSIMDEKNTPIRTYQVCNVMEPSQNNWLRTDWITREGAQRVYIEIKFTLRDCNSLPGVMGTCKETFNLYYYESDNDKERFIRENQFVKIDTIAADESFTQVDIGDRIMKLNTEIRDVGPLSKKGFYLAFQDVGACIALVSVRVFYKKCPLTVRNLAQFPDTITGADTSSLVEVRGSCVNNSEEKDVPKMYCGADGEWLVPIGNCLCNAGHEERSGECQACKIGYYKALSTDATCAKCPPHSYSVWEGATSCTCDRGFFRADNDAASMPCTRPPSAPLNLISNVNETSVNLEWSSPQNTGGRQDISYNVVCKKCGAGDPSKCRPCGSGVHYTPQQNGLKTTKVSITDLLAHTNYTFEIWAVNGVSKYNPNPDQSVSVTVTTNQAAPSSIALVQAKEVTRYSVALAWLEPDRPNGVILEYEVKYYEKDQNERSYRIVRTAARNTDIKGLNPLTSYVFHVRARTAAGYGDFSEPLEVTTNTVPSRIIGDGANSTAAAHHHHHHHHHH

SEQ ID NO: 5 - protein, 905 aa, synthetic construct
  REGION 1..905: note = Synthetic polypeptide
VTGSRVYPANEVTLLDSRSVQGELGWIASPLEGGWEEVSIMDEKNTPIRTYQVCNVMEPSQNNWLRTDWITREGAQRVYIEIKFTLRDCNSLPGVMGTCKETFNLYYYESDNDKERFIRENQFVKIDTIAADESFTQVDIGDRIMKLNTEIRDVGPLSKKGFYLAFQDVGACIALVSVRVFYKKCPLTVRNLAQFPDTITGADTSSLVEVRGSCVNNSEEKDVPKMYCGADGEWLVPIGNCLCNAGHEERSGECQACKIGYYKALSTDATCAKCPPHSYSVWEGATSCTCDRGFFRADNDAASMPCTRPPSAPLNLISNVNETSVNLEWSSPQNTGGRQDISYNVVCKKCGAGDPSKCRPCGSGVHYTPQQNGLKTTKVSITDLLAHTNYTFEIWAVNGVSKYNPNPDQSVSVTVTTNQAAPSSIALVQAKEVTRYSVALAWLEPDRPNGVILEYEVKYYEKDQNERSYRIVRTAARNTDIKGLNPLTSYVFHVRARTAAGYGDFSEPLEVTTNTVPSRIIGDGANSTAAAEEGKLVIWINGDKGYNGLAEVGKKFEKDTGIKVTVEHPDKLEEKFPQVAATGDGPDIIFWAHDRFGGYAQSGLLAEITPDKAFQDKLYPFTWDAVRYNGKLIAYPIAVEALSLIYNKDLLPNPPKTWEEIPALDKELKAKGKSALMFNLQEPYFTWPLIAADGGYAFKYENGKYDIKDVGVDNAGAKAGLTFLVDLIKNKHMNADTDYSIAEAAFNKGETAMTINGPWAWSNIDTSKVNYGVTVLPTFKGQPSKPFVGVLSAGINAASPNKELAKEFLENYLLTDEGLEAVNKDKPLGAVALKSYEEELAKDPRIAATMENAQKGEIMPNIPQMSAFWYAVRTAVINAASGRQTVDEALKDAQTHHHHHHHHHH

SEQ ID NO: 6 - protein, 119 aa, synthetic construct
  REGION 1..119: note = Synthetic polypeptide
QEQLKESGGRLVTPGGSLTLTCTVSGIDLSSYAMSWVRQAPEKGLEWIGFINMYGTYYASWAKGRFTISRTSTTVDLKVTSLTTEDTATYFCVRGGRSPDYDIVSGDIWGPGTLVTVSS

SEQ ID NO: 7 - protein, 110 aa, synthetic construct
  REGION 1..110: note = Synthetic polypeptide
YVMMTQTPSSVSEPVGGTVTIKCQASQNIYNSLAWYQQKPGQRPKLLIADASELASGVPQRFSGSGSGTQFTLTISDLECADAATYYCQSSSAGDSYVGGFGGGTEVVVK

SEQ ID NO: 8 - DNA, 357 bp, synthetic construct
  misc_feature 1..357: note = Synthetic oligonucleotide
  source 1..357: mol_type = other DNA
caggagcagctgaaggagtccgggggtcgcctggtaacgcctggaggatccctgacactcacctgcacagtctctggaatcgacctcagtagctatgcaatgagctgggtccgccaggctccagagaaggggctggaatggatcggattcattaatatgtatggtacatactacgcgagctgggcgaaaggccgattcaccatctccagaacctcgaccacggtggatctgaaagtgaccagtctgacaaccgaggacacggccacctatttctgtgtcagagggggcaggtctcctgattatgatattgttagtggggacatctggggcccaggcaccctggtcaccgtctcttca

SEQ ID NO: 9 - DNA, 330 bp, synthetic construct
  misc_feature 1..330: note = Synthetic oligonucleotide
  source 1..330: mol_type = other DNA
tatgtcatgatgacccagactccatcctccgtgtctgaacctgtgggaggcacagtcaccatcaagtgccaggccagtcagaacatttacaactctttagcctggtatcagcagaaaccaggacagcgtcccaagctcctgatcgccgatgcatcggaactggcatctggggtcccacagcggttcagcggcagtggatctgggacacagttcactctcaccatcagcgacctggagtgtgccgatgctgccacttactactgtcagtctagtagtgctggtgatagttatgttggtggtttcggcggagggaccgaggtggtggtcaaa

SEQ ID NO: 10 - protein, 115 aa, synthetic construct
  REGION 1..115: note = Synthetic polypeptide
QSLEESGGRLVTPGTPLTLTCTVSGFSLSSYHMSWVRQAPGKGLEWIGIIYRSGNTYYANWAKGRFTISKTSTTVDLKITSPTTEDTATYFCARESSTFYGMDLWGPGTLVTVSS

SEQ ID NO: 11 - protein, 109 aa, synthetic construct
  REGION 1..109: note = Synthetic polypeptide
DPVLTQTASSVSAAVGGTVTINCQASQSVYGNNELAWYQQKPGQPPKLLIYTASSLASGVPSRFKGSGSGTEFTLTISDLECADAATYYCLGYKSDDYTFGGGTEVVVK

SEQ ID NO: 12 - DNA, 345 bp, synthetic construct
  misc_feature 1..345: note = Synthetic oligonucleotide
  source 1..345: mol_type = other DNA
cagtcgttggaggagtccgggggtcgcctggtcacgcctgggacacccctgacactcacctgcacagtctctggattctccctcagcagctaccacatgagctgggtccgccaggctccagggaaggggctggagtggatcggaattatttataggagtggtaatacatactacgcgaactgggcgaaaggccgattcaccatctccaaaacctcgaccacggtggatctgaaaatcaccagtccgacaaccgaggacacggccacctatttctgtgccagagaaagtagtactttctacggcatggacctctggggcccagggaccctcgtcaccgtctcttca

SEQ ID NO: 13 - DNA, 327 bp, synthetic construct
  misc_feature 1..327: note = Synthetic oligonucleotide
  source 1..327: mol_type = other DNA
gaccctgtgctgacccagactgcatcctccgtgtctgcagctgtgggaggcacagtcaccatcaattgccaggccagtcagagtgtttatggtaacaacgaattagcctggtatcagcagaaaccagggcagcctcccaagctcctgatctatactgcatccagtctggcatctggggtcccatcgcggttcaaaggcagtggatctgggacagagttcactctcaccatcagcgacctggagtgtgccgatgctgccacttactactgcctaggttataaaagtgatgactatactttcggcggagggaccgaggtggtggtcaaa

SEQ ID NO: 14 - protein, 115 aa, synthetic construct; identical to SEQ ID NO: 10
  REGION 1..115: note = Synthetic polypeptide

SEQ ID NO: 15 - protein, 109 aa, synthetic construct
  REGION 1..109: note = Synthetic polypeptide
AIKMTQTPSSVSAAVGGTVTINCQASQSVYGNNELAWYQQKPGQPPKLLIYTASSLASGVPSRFKGSGSGTEFTLTISDLECADAATYYCLGYKSDDYTFGGGTEVVVK

SEQ ID NO: 16 - DNA, 345 bp, synthetic construct
  misc_feature 1..345: note = Synthetic oligonucleotide
  source 1..345: mol_type = other DNA
cagtcgctggaggagtccgggggtcgcctggtcacgcctgggacacccctgacactcacctgcacagtctctggattctccctcagcagctaccacatgagctgggtccgccaggctccagggaaggggctggagtggatcggaattatttataggagtggtaatacatactacgcgaactgggcgaaaggccgattcaccatctccaaaacctcgaccacggtggatctgaaaatcaccagtccgacaaccgaggacacggccacctatttctgtgccagagaaagtagtactttctacggcatggacctctggggcccagggaccctcgtcaccgtctcttca

SEQ ID NO: 17 - DNA, 327 bp, synthetic construct
  misc_feature 1..327: note = Synthetic oligonucleotide
  source 1..327: mol_type = other DNA
gccattaaaatgacccagactccatcctccgtgtctgcagctgtgggaggcacagtcaccatcaattgccaggccagtcagagtgtttatggtaacaacgaattagcctggtatcagcagaaaccagggcagcctcccaagctcctgatctatactgcatccagtctggcatctggggtcccatcgcggttcaaaggcagtggatctgggacagagttcactctcaccatcagcgacctggagtgtgccgatgctgccacttactactgcctaggttataaaagtgatgactatactttcggcggagggaccgaggtggtagtcaaa

SEQ ID NO: 18 - protein, 118 aa, synthetic construct
  REGION 1..118: note = Synthetic polypeptide
QSLEESGGRLVTPGTPLTLTCTISGFSLSSFYINWVRQAPGRGLEWIGIIYPDIDATDYASWVKGRFTISKTSTTVDLKITSPTTEDTATYFCARSDVDYYTTRLDLWGQGTLVTVSS

SEQ ID NO: 19 - protein, 110 aa, synthetic construct
  REGION 1..110: note = Synthetic polypeptide
DPMMTQTASPVSAAVGGTVSISCQSNKSVYSNWLSWFQQKPGQPPKLLIYGASTLASGVPSRFKGSGSGTQFTLTVSDVQCDDAATYFCLGGYRDNSDNAFGGGTEVVVK

SEQ ID NO: 20 - DNA, 354 bp, synthetic construct
  misc_feature 1..354: note = Synthetic oligonucleotide
  source 1..354: mol_type = other DNA
cagtcgttggaggagtccgggggtcgcctggtcacgcctgggacacccctgacactcacctgcacaatctctggattctccctcagtagcttctacataaactgggtccgccaggctccagggagggggctggaatggatcggaatcatttatcctgatattgatgccacagactacgcgagctgggtgaaaggccgattcaccatctccaaaacctcgaccacggtggatctgaaaatcaccagtccgacaaccgaggacacggccacctatttctgtgccagaagtgatgttgattattatacaactcggttggatctctggggccagggcaccctggtcaccgtctcctca

SEQ ID NO: 21 - DNA, 330 bp, synthetic construct
  misc_feature 1..330: note = Synthetic oligonucleotide
  source 1..330: mol_type = other DNA
gaccctatgatgacccagactgcatctcccgtgtctgcagctgtgggaggcacagtcagcatcagttgccagtccaataagagtgtttatagtaactggttatcctggtttcagcagaaaccagggcagcctcccaagctcctgatctatggtgcatccactctggcatctggggtcccatcgcggttcaaaggcagtggatctgggacacagttcactctcaccgtcagcgacgtgcagtgtgacgatgctgccacttacttctgtctaggcggttatcgtgataatagtgataatgctttcggcggagggaccgaggtggtggtcaaa

SEQ ID NO: 22 - protein, 323 aa, Oryctolagus cuniculus
GAPKAPSVFPLAPCCGDTPSSTVTLGCLVKGYLPEPVTVTWNSGTLTNGVRTFPSVRQSSGLYSLSSVVSVTSSSQPVTCNVAHPATNTKVDKTVAPSTCSKPTCPPPELLGGPSVFIFPPKPKDTLMISRTPEVTCVVVDVSQDDPEVQFTWYINNEQVRTARPPLREQQFNSTIRVVSTLPITHQDWLRGKEFKCKVHNKALPAPIEKTISKARGQPLEPKVYTMGPPREELSSRSVSLTCMINGFYPSDISVEWEKNGKAEDNYKTTPAVLDSDGSYFLYNKLSVPTSEWQRGDVFTCSVMHEALHNHYTQKSISRSPGK

SEQ ID NO: 23 - protein, 104 aa, Oryctolagus cuniculus
GAPVAPTVLIFPPAADQVATGTVTIVCVANKYFPDVTVTWEVDGTTQTTGIENSKTPQNSADCTYNLSSTLTLTSTQYNSHKEYTCKVTQGTTSVVQSFNRGDC

SEQ ID NO: 24 - protein, 442 aa, synthetic construct
  REGION 1..442: note = Synthetic polypeptide
QEQLKESGGRLVTPGGSLTLTCTVSGIDLSSYAMSWVRQAPEKGLEWIGFINMYGTYYASWAKGRFTISRTSTTVDLKVTSLTTEDTATYFCVRGGRSPDYDIVSGDIWGPGTLVTVSSGAPKAPSVFPLAPCCGDTPSSTVTLGCLVKGYLPEPVTVTWNSGTLTNGVRTFPSVRQSSGLYSLSSVVSVTSSSQPVTCNVAHPATNTKVDKTVAPSTCSKPTCPPPELLGGPSVFIFPPKPKDTLMISRTPEVTCVVVDVSQDDPEVQFTWYINNEQVRTARPPLREQQFNSTIRVVSTLPITHQDWLRGKEFKCKVHNKALPAPIEKTISKARGQPLEPKVYTMGPPREELSSRSVSLTCMINGFYPSDISVEWEKNGKAEDNYKTTPAVLDSDGSYFLYNKLSVPTSEWQRGDVFTCSVMHEALHNHYTQKSISRSPGK

SEQ ID NO: 25 - protein, 214 aa, synthetic construct
  REGION 1..214: note = Synthetic polypeptide
YVMMTQTPSSVSEPVGGTVTIKCQASQNIYNSLAWYQQKPGQRPKLLIADASELASGVPQRFSGSGSGTQFTLTISDLECADAATYYCQSSSAGDSYVGGFGGGTEVVVKGAPVAPTVLIFPPAADQVATGTVTIVCVANKYFPDVTVTWEVDGTTQTTGIENSKTPQNSADCTYNLSSTLTLTSTQYNSHKEYTCKVTQGTTSVVQSFNRGDC

SEQ ID NO: 26 - DNA, 1326 bp, synthetic construct
  misc_feature 1..1326: note = Synthetic oligonucleotide
  source 1..1326: mol_type = other DNA
caggagcagctgaaggagtccgggggtcgcctggtaacgcctggaggatccctgacactcacctgcacagtctctggaatcgacctcagtagctatgcaatgagctgggtccgccaggctccagagaaggggctggaatggatcggattcattaatatgtatggtacatactacgcgagctgggcgaaaggccgattcaccatctccagaacctcgaccacggtggatctgaaagtgaccagtctgacaaccgaggacacggccacctatttctgtgtcagagggggcaggtctcctgattatgatattgttagtggggacatctggggcccaggcaccctggtcaccgtctcttcaggggccccaaaggccccaagcgtgttccctctggctccatgctgtggcgacacacccagctccaccgtgacactgggctgcctggtgaagggctacctgcccgagcctgtgaccgtgacatggaactccggcaccctgacaaatggcgtgagaacctttccttctgtgcgccagtctagcggcctgtatagcctgtcctctgtggtgtccgtgacaagctcctctcagcctgtgacctgtaacgtggcccacccagctaccaatacaaaggtggataagaccgtggccccatccacatgctctaagcccacctgtccacctccagagctgctgggaggaccatccgtgttcatctttccccctaagcctaaggacacactgatgatcagccggacccctgaggtgacatgcgtggtggtggacgtgagccaggacgatccagaggtgcagttcacatggtacatcaacaatgagcaggtgcggaccgccaggccacccctgagagagcagcagtttaactctaccatccgcgtggtgagcaccctgccaatcacacaccaggactggctgagaggcaaggagttcaagtgcaaggtgcacaataaggccctgccagctcccatcgagaagacaatctctaaggctaggggacagccactggagcctaaggtgtataccatgggacctccaagggaggagctgagctccaggtctgtgagcctgacctgtatgatcaacggcttttaccccagcgacatctccgtggagtgggagaagaacggcaaggccgaggataattataagaccacacccgctgtgctggactctgatggcagctacttcctgtataacaagctgtccgtgcctacatctgagtggcagcggggcgacgtgttcacctgttccgtgatgcacgaggctctgcacaatcactacacccagaagtccatctctaggagccccggcaag

SEQ ID NO: 27 - DNA, 642 bp, synthetic construct
  misc_feature 1..642: note = Synthetic oligonucleotide
  source 1..642: mol_type = other DNA
tatgtcatgatgacccagactccatcctccgtgtctgaacctgtgggaggcacagtcaccatcaagtgccaggccagtcagaacatttacaactctttagcctggtatcagcagaaaccaggacagcgtcccaagctcctgatcgccgatgcatcggaactggcatctggggtcccacagcggttcagcggcagtggatctgggacacagttcactctcaccatcagcgacctggagtgtgccgatgctgccacttactactgtcagtctagtagtgctggtgatagttatgttggtggtttcggcggagggaccgaggtggtggtcaaaggggccccagtggccccaaccgtgctgatcttcccacctgctgctgaccaggtggctaccggaacagtgaccatcgtgtgcgtggctaacaagtactttccagacgtgacagtgacctgggaggtggatggcaccacacagaccacaggcatcgagaacagcaagacaccccagaacagcgccgactgtacctataacctgagctccacactgaccctgacatccacccagtacaattctcacaaggagtatacatgcaaggtgacacagggcaccacatctgtggtgcagagcttcaatcggggcgattgt

SEQ ID NO: 28 - protein, 438 aa, synthetic construct
  REGION 1..438: note = Synthetic polypeptide
QSLEESGGRLVTPGTPLTLTCTVSGFSLSSYHMSWVRQAPGKGLEWIGIIYRSGNTYYANWAKGRFTISKTSTTVDLKITSPTTEDTATYFCARESSTFYGMDLWGPGTLVTVSSGAPKAPSVFPLAPCCGDTPSSTVTLGCLVKGYLPEPVTVTWNSGTLTNGVRTFPSVRQSSGLYSLSSVVSVTSSSQPVTCNVAHPATNTKVDKTVAPSTCSKPTCPPPELLGGPSVFIFPPKPKDTLMISRTPEVTCVVVDVSQDDPEVQFTWYINNEQVRTARPPLREQQFNSTIRVVSTLPITHQDWLRGKEFKCKVHNKALPAPIEKTISKARGQPLEPKVYTMGPPREELSSRSVSLTCMINGFYPSDISVEWEKNGKAEDNYKTTPAVLDSDGSYFLYNKLSVPTSEWQRGDVFTCSVMHEALHNHYTQKSISRSPGK

SEQ ID NO: 29 - protein, 213 aa, synthetic construct
  REGION 1..213: note = Synthetic polypeptide
DPVLTQTASSVSAAVGGTVTINCQASQSVYGNNELAWYQQKPGQPPKLLIYTASSLASGVPSRFKGSGSGTEFTLTISDLECADAATYYCLGYKSDDYTFGGGTEVVVKGAPVAPTVLIFPPAADQVATGTVTIVCVANKYFPDVTVTWEVDGTTQTTGIENSKTPQNSADCTYNLSSTLTLTSTQYNSHKEYTCKVTQGTTSVVQSFNRGDC

SEQ ID NO: 30 - DNA, 1314 bp, synthetic construct
  misc_feature 1..1314: note = Synthetic oligonucleotide
  source 1..1314: mol_type = other DNA
cagtcgttggaggagtccgggggtcgcctggtcacgcctgggacacccctgacactcacctgcacagtctctggattctccctcagcagctaccacatgagctgggtccgccaggctccagggaaggggctggagtggatcggaattatttataggagtggtaatacatactacgcgaactgggcgaaaggccgattcaccatctccaaaacctcgaccacggtggatctgaaaatcaccagtccgacaaccgaggacacggccacctatttctgtgccagagaaagtagtactttctacggcatggacctctggggcccagggaccctcgtcaccgtctcttcaggggccccaaaggccccaagcgtgttccctctggctccatgctgtggcgacacacccagctccaccgtgacactgggctgcctggtgaagggctacctgcccgagcctgtgaccgtgacatggaactccggcaccctgacaaatggcgtgagaacctttccttctgtgcgccagtctagcggcctgtatagcctgtcctctgtggtgtccgtgacaagctcctctcagcctgtgacctgtaacgtggcccacccagctaccaatacaaaggtggataagaccgtggccccatccacatgctctaagcccacctgtccacctccagagctgctgggaggaccatccgtgttcatctttccccctaagcctaaggacacactgatgatcagccggacccctgaggtgacatgcgtggtggtggacgtgagccaggacgatccagaggtgcagttcacatggtacatcaacaatgagcaggtgcggaccgccaggccacccctgagagagcagcagtttaactctaccatccgcgtggtgagcaccctgccaatcacacaccaggactggctgagaggcaaggagttcaagtgcaaggtgcacaataaggccctgccagctcccatcgagaagacaatctctaaggctaggggacagccactggagcctaaggtgtataccatgggacctccaagggaggagctgagctccaggtctgtgagcctgacctgtatgatcaacggcttttaccccagcgacatctccgtggagtgggagaagaacggcaaggccgaggataattataagaccacacccgctgtgctggactctgatggcagctacttcctgtataacaagctgtccgtgcctacatctgagtggcagcggggcgacgtgttcacctgttccgtgatgcacgaggctctgcacaatcactacacccagaagtccatctctaggagccccggcaag

SEQ ID NO: 31 - DNA, 639 bp, synthetic construct
  misc_feature 1..639: note = Synthetic oligonucleotide
  source 1..639: mol_type = other DNA
gaccctgtgctgacccagactgcatcctccgtgtctgcagctgtgggaggcacagtcaccatcaattgccaggccagtcagagtgtttatggtaacaacgaattagcctggtatcagcagaaaccagggcagcctcccaagctcctgatctatactgcatccagtctggcatctggggtcccatcgcggttcaaaggcagtggatctgggacagagttcactctcaccatcagcgacctggagtgtgccgatgctgccacttactactgcctaggttataaaagtgatgactatactttcggcggagggaccgaggtggtggtcaaaggggccccagtggccccaaccgtgctgatcttcccacctgctgctgaccaggtggctaccggaacagtgaccatcgtgtgcgtggctaacaagtactttccagacgtgacagtgacctgggaggtggatggcaccacacagaccacaggcatcgagaacagcaagacaccccagaacagcgccgactgtacctataacctgagctccacactgaccctgacatccacccagtacaattctcacaaggagtatacatgcaaggtgacacagggcaccacatctgtggtgcagagcttcaatcggggcgattgt

SEQ ID NO: 32 - protein, 438 aa, synthetic construct; identical to SEQ ID NO: 28
  REGION 1..438: note = Synthetic polypeptide

SEQ ID NO: 33 - protein, 213 aa, synthetic construct
  REGION 1..213: note = Synthetic polypeptide
AIKMTQTPSSVSAAVGGTVTINCQASQSVYGNNELAWYQQKPGQPPKLLIYTASSLASGVPSRFKGSGSGTEFTLTISDLECADAATYYCLGYKSDDYTFGGGTEVVVKGAPVAPTVLIFPPAADQVATGTVTIVCVANKYFPDVTVTWEVDGTTQTTGIENSKTPQNSADCTYNLSSTLTLTSTQYNSHKEYTCKVTQGTTSVVQSFNRGDC

SEQ ID NO: 34 - DNA, 1314 bp, synthetic construct
  misc_feature 1..1314: note = Synthetic oligonucleotide
  source 1..1314: mol_type = other DNA
cagtcgctggaggagtccgggggtcgcctggtcacgcctgggacacccctgacactcacctgcacagtctctggattctccctcagcagctaccacatgagctgggtccgccaggctccagggaaggggctggagtggatcggaattatttataggagtggtaatacatactacgcgaactgggcgaaaggccgattcaccatctccaaaacctcgaccacggtggatctgaaaatcaccagtccgacaaccgaggacacggccacctatttctgtgccagagaaagtagtactttctacggcatggacctctggggcccagggaccctcgtcaccgtctcttcaggggccccaaaggccccaagcgtgttccctctggctccatgctgtggcgacacacccagctccaccgtgacactgggctgcctggtgaagggctacctgcccgagcctgtgaccgtgacatggaactccggcaccctgacaaatggcgtgagaacctttccttctgtgcgccagtctagcggcctgtatagcctgtcctctgtggtgtccgtgacaagctcctctcagcctgtgacctgtaacgtggcccacccagctaccaatacaaaggtggataagaccgtggccccatccacatgctctaagcccacctgtccacctccagagctgctgggaggaccatccgtgttcatctttccccctaagcctaaggacacactgatgatcagccggacccctgaggtgacatgcgtggtggtggacgtgagccaggacgatccagaggtgcagttcacatggtacatcaacaatgagcaggtgcggaccgccaggccacccctgagagagcagcagtttaactctaccatccgcgtggtgagcaccctgccaatcacacaccaggactggctgagaggcaaggagttcaagtgcaaggtgcacaataaggccctgccagctcccatcgagaagacaatctctaaggctaggggacagccactggagcctaaggtgtataccatgggacctccaagggaggagctgagctccaggtctgtgagcctgacctgtatgatcaacggcttttaccccagcgacatctccgtggagtgggagaagaacggcaaggccgaggataattataagaccacacccgctgtgctggactctgatggcagctacttcctgtataacaagctgtccgtgcctacatctgagtggcagcggggcgacgtgttcacctgttccgtgatgcacgaggctctgcacaatcactacacccagaagtccatctctaggagccccggcaag

SEQ ID NO: 35 - DNA, 639 bp, synthetic construct
  misc_feature 1..639: note = Synthetic oligonucleotide
  source 1..639: mol_type = other DNA
gccattaaaatgacccagactccatcctccgtgtctgcagctgtgggaggcacagtcaccatcaattgccaggccagtcagagtgtttatggtaacaacgaattagcctggtatcagcagaaaccagggcagcctcccaagctcctgatctatactgcatccagtctggcatctggggtcccatcgcggttcaaaggcagtggatctgggacagagttcactctcaccatcagcgacctggagtgtgccgatgctgccacttactactgcctaggttataaaagtgatgactatactttcggcggagggaccgaggtggtagtcaaaggggccccagtggccccaaccgtgctgatcttcccacctgctgctgaccaggtggctaccggaacagtgaccatcgtgtgcgtggctaacaagtactttccagacgtgacagtgacctgggaggtggatggcaccacacagaccacaggcatcgagaacagcaagacaccccagaacagcgccgactgtacctataacctgagctccacactgaccctgacatccacccagtacaattctcacaaggagtatacatgcaaggtgacacagggcaccacatctgtggtgcagagcttcaatcggggcgattgt

SEQ ID NO: 36 - protein, 441 aa, synthetic construct
  REGION 1..441: note = Synthetic polypeptide
QSLEESGGRLVTPGTPLTLTCTISGFSLSSFYINWVRQAPGRGLEWIGIIYPDIDATDYASWVKGRFTISKTSTTVDLKITSPTTEDTATYFCARSDVDYYTTRLDLWGQGTLVTVSSGAPKAPSVFPLAPCCGDTPSSTVTLGCLVKGYLPEPVTVTWNSGTLTNGVRTFPSVRQSSGLYSLSSVVSVTSSSQPVTCNVAHPATNTKVDKTVAPSTCSKPTCPPPELLGGPSVFIFPPKPKDTLMISRTPEVTCVVVDVSQDDPEVQFTWYINNEQVRTARPPLREQQFNSTIRVVSTLPITHQDWLRGKEFKCKVHNKALPAPIEKTISKARGQPLEPKVYTMGPPREELSSRSVSLTCMINGFYPSDISVEWEKNGKAEDNYKTTPAVLDSDGSYFLYNKLSVPTSEWQRGDVFTCSVMHEALHNHYTQKSISRSPGK

SEQ ID NO: 37 - protein, 214 aa, synthetic construct
  REGION 1..214: note = Synthetic polypeptide
DPMMTQTASPVSAAVGGTVSISCQSNKSVYSNWLSWFQQKPGQPPKLLIYGASTLASGVPSRFKGSGSGTQFTLTVSDVQCDDAATYFCLGGYRDNSDNAFGGGTEVVVKGAPVAPTVLIFPPAADQVATGTVTIVCVANKYFPDVTVTWEVDGTTQTTGIENSKTPQNSADCTYNLSSTLTLTSTQYNSHKEYTCKVTQGTTSVVQSFNRGDC

SEQ ID NO: 38 - DNA, 1323 bp, synthetic construct
  misc_feature 1..1323: note = Synthetic oligonucleotide
  source 1..1323: mol_type = other DNA
cagtcgttggaggagtccgggggtcgcctggtcacgcctgggacacccctgacactcacctgcacaatctctggattctccctcagtagcttctacataaactgggtccgccaggctccagggagggggctggaatggatcggaatcatttatcctgatattgatgccacagactacgcgagctgggtgaaaggccgattcaccatctccaaaacctcgaccacggtggatctgaaaatcaccagtccgacaaccgaggacacggccacctatttctgtgccagaagtgatgttgattattatacaactcggttggatctctggggccagggcaccctggtcaccgtctcctcaggggccccaaaggccccaagcgtgttccctctggctccatgctgtggcgacacacccagctccaccgtgacactgggctgcctggtgaagggctacctgcccgagcctgtgaccgtgacatggaactccggcaccctgacaaatggcgtgagaacctttccttctgtgcgccagtctagcggcctgtatagcctgtcctctgtggtgtccgtgacaagctcctctcagcctgtgacctgtaacgtggcccacccagctaccaatacaaaggtggataagaccgtggccccatccacatgctctaagcccacctgtccacctccagagctgctgggaggaccatccgtgttcatctttccccctaagcctaaggacacactgatgatcagccggacccctgaggtgacatgcgtggtggtggacgtgagccaggacgatccagaggtgcagttcacatggtacatcaacaatgagcaggtgcggaccgccaggccacccctgagagagcagcagtttaactctaccatccgcgtggtgagcaccctgccaatcacacaccaggactggctgagaggcaaggagttcaagtgcaaggtgcacaataaggccctgccagctcccatcgagaagacaatctctaaggctaggggacagccactggagcctaaggtgtataccatgggacctccaagggaggagctgagctccaggtctgtgagcctgacctgtatgatcaacggcttttaccccagcgacatctccgtggagtgggagaagaacggcaaggccgaggataattataagaccacacccgctgtgctggactctgatggcagctacttcctgtataacaagctgtccgtgcctacatctgagtggcagcggggcgacgtgttcacctgttccgtgatgcacgaggctctgcacaatcactacacccagaagtccatctctaggagccccggcaag

SEQ ID NO: 39 - DNA, 642 bp, synthetic construct
  misc_feature 1..642: note = Synthetic oligonucleotide
  source 1..642: mol_type = other DNA
gaccctatgatgacccagactgcatctcccgtgtctgcagctgtgggaggcacagtcagcatcagttgccagtccaataagagtgtttatagtaactggttatcctggtttcagcagaaaccagggcagcctcccaagctcctgatctatggtgcatccactctggcatctggggtcccatcgcggttcaaaggcagtggatctgggacacagttcactctcaccgtcagcgacgtgcagtgtgacgatgctgccacttacttctgtctaggcggttatcgtgataatagtgataatgctttcggcggagggaccgaggtggtggtcaaaggggccccagtggccccaaccgtgctgatcttcccacctgctgctgaccaggtggctaccggaacagtgaccatcgtgtgcgtggctaacaagtactttccagacgtgacagtgacctgggaggtggatggcaccacacagaccacaggcatcgagaacagcaagacaccccagaacagcgccgactgtacctataacctgagctccacactgaccctgacatccacccagtacaattctcacaaggagtatacatgcaaggtgacacagggcaccacatctgtggtgcagagcttcaatcggggcgattgt

SEQ ID NO: 40 - protein, 5 aa, synthetic construct
  REGION 1..5: note = Synthetic polypeptide
SYAMS

SEQ ID NO: 41 - protein, 15 aa, synthetic construct
  REGION 1..15: note = Synthetic polypeptide
FINMYGTYYASWAKG

SEQ ID NO: 42 - protein, 14 aa, synthetic construct
  REGION 1..14: note = Synthetic polypeptide
GGRSPDYDIVSGDI

SEQ ID NO: 43 - protein, 11 aa, synthetic construct
  REGION 1..11: note = Synthetic polypeptide
QASQNIYNSLA

SEQ ID NO: 44 - protein, 7 aa, synthetic construct
  REGION 1..7: note = Synthetic polypeptide
DASELAS

SEQ ID NO: 45 - protein, 12 aa, synthetic construct
  REGION 1..12: note = Synthetic polypeptide
QSSSAGDSYVGG

SEQ ID NO: 46 - DNA, 15 bp, synthetic construct
  misc_feature 1..15: note = Synthetic oligonucleotide
  source 1..15: mol_type = other DNA
agctatgcaatgagc

SEQ ID NO: 47 - DNA, 45 bp, synthetic construct
  misc_feature 1..45: note = Synthetic oligonucleotide
  source 1..45: mol_type = other DNA
ttcattaatatgtatggtacatactacgcgagctgggcgaaaggc

SEQ ID NO: 48 - DNA, 42 bp, synthetic construct
  misc_feature 1..42: note = Synthetic oligonucleotide
  source 1..42: mol_type = other DNA
gggggcaggtctcctgattatgatattgttagtggggacatc

SEQ ID NO: 49 - DNA, 33 bp, synthetic construct
  misc_feature 1..33: note = Synthetic oligonucleotide
  source 1..33: mol_type = other DNA
caggccagtcagaacatttacaactctttagcc

SEQ ID NO: 50 - DNA, 22 bp, synthetic construct
  misc_feature 1..22: note = Synthetic oligonucleotide
  source 1..22: mol_type = other DNA
gatgcatcggaactggcatctg

SEQ ID NO: 51 - DNA, 36 bp, synthetic construct
  misc_feature 1..36: note = Synthetic oligonucleotide
  source 1..36: mol_type = other DNA
cagtctagtagtgctggtgatagttatgttggtggt

SEQ ID NO: 52 - protein, 5 aa, synthetic construct
  REGION 1..5: note = Synthetic polypeptide
SYHMS

SEQ ID NO: 53 - protein, 16 aa, synthetic construct
  REGION 1..16: note = Synthetic polypeptide
IIYRSGNTYYANWAKG

SEQ ID NO: 54 - protein, 10 aa, synthetic construct
  REGION 1..10: note = Synthetic polypeptide
ESSTFYGMDL

SEQ ID NO: 55 - protein, 13 aa, synthetic construct
  REGION 1..13: note = Synthetic polypeptide
QASQSVYGNNELA

SEQ ID NO: 56 - protein, 7 aa, synthetic construct
  REGION 1..7: note = Synthetic polypeptide
TASSLAS

SEQ ID NO: 57 - protein, 9 aa, synthetic construct
  REGION 1..9: note = Synthetic polypeptide
LGYKSDDYT

SEQ ID NO: 58 - DNA, 15 bp, synthetic construct
  misc_feature 1..15: note = Synthetic oligonucleotide
  source 1..15: mol_type = other DNA
agctaccacatgagc

SEQ ID NO: 59 - DNA, 48 bp, synthetic construct
  misc_feature 1..48: note = Synthetic oligonucleotide
  source 1..48: mol_type = other DNA
attatttataggagtggtaatacatactacgcgaactgggcgaaaggc

SEQ ID NO: 60 - DNA, 30 bp, synthetic construct
  misc_feature 1..30: note = Synthetic oligonucleotide
  source 1..30: mol_type = other DNA
gaaagtagtactttctacggcatggacctc

SEQ ID NO: 61 - DNA, 39 bp, synthetic construct
  misc_feature 1..39: note = Synthetic oligonucleotide
  source 1..39: mol_type = other DNA
caggccagtcagagtgtttatggtaacaacgaattagcc

SEQ ID NO: 62 - DNA, 21 bp, synthetic construct
  misc_feature 1..21: note = Synthetic oligonucleotide
  source 1..21: mol_type = other DNA
actgcatccagtctggcatct

SEQ ID NO: 63 - DNA, 27 bp, synthetic construct
  misc_feature 1..27: note = Synthetic oligonucleotide
  source 1..27: mol_type = other DNA
ctaggttataaaagtgatgactatact

SEQ ID NO: 64 - protein, 5 aa, synthetic construct
  REGION 1..5: note = Synthetic polypeptide
SFYIN

SEQ ID NO: 65 - protein, 17 aa, synthetic construct
  REGION 1..17: note = Synthetic polypeptide
IIYPDIDATDYASWVKG

SEQ ID NO: 66 - protein, 12 aa, synthetic construct
  REGION 1..12: note = Synthetic polypeptide
SDVDYYTTRLDL

SEQ ID NO: 67 - protein, 12 aa, synthetic construct
  REGION 1..12: note = Synthetic polypeptide
QSNKSVYSNWLS

SEQ ID NO: 68 - protein, 7 aa, synthetic construct
  REGION 1..7: note = Synthetic polypeptide
GASTLAS

SEQ ID NO: 69 - protein, 11 aa, synthetic construct
  REGION 1..11: note = Synthetic polypeptide
LGGYRDNSDNA

SEQ ID NO: 70 - DNA, 15 bp, synthetic construct
  misc_feature 1..15: note = Synthetic oligonucleotide
  source 1..15: mol_type = other DNA
agcttctacataaac

SEQ ID NO: 71 - DNA, 51 bp, synthetic construct
  misc_feature 1..51: note = Synthetic oligonucleotide
  source 1..51: mol_type = other DNA
atcatttatcctgatattgatgccacagactacgcgagctgggtgaaaggc

SEQ ID NO: 72 - DNA, 36 bp, synthetic construct
  misc_feature 1..36: note = Synthetic oligonucleotide
  source 1..36: mol_type = other DNA
agtgatgttgattattatacaactcggttggatctc

SEQ ID NO: 73 - DNA, 36 bp, synthetic construct
  misc_feature 1..36: note = Synthetic oligonucleotide
  source 1..36: mol_type = other DNA
cagtccaataagagtgtttatagtaactggttatcc

SEQ ID NO: 74 - DNA, 21 bp, synthetic construct
  misc_feature 1..21: note = Synthetic oligonucleotide
  source 1..21: mol_type = other DNA
ggtgcatccactctggcatct

SEQ ID NO: 75 - DNA, 33 bp, synthetic construct
  misc_feature 1..33: note = Synthetic oligonucleotide
  source 1..33: mol_type = other DNA
ctaggcggttatcgtgataatagtgataatgct

SEQ ID NO: 76 - protein, 115 aa, synthetic construct
  REGION 1..115: note = Synthetic polypeptide
QSVEESGGRLVTPGTPLTLTCTVSGFSLSSYHMSWVRQAPGKGLEWIGIIYRSGNTYSANWAKGRFTISKTSTTVDLKITSPTTEDTATYFCARESSTFYGMDLWGPGTLVTVSS

SEQ ID NO: 77 - protein, 109 aa, synthetic construct
  REGION 1..109: note = Synthetic polypeptide
YVMMTQTPSSVSAAVGGTVTINCQASQSVYGNNELAWYQQKPGQRPKLLIYRASTLASGVPSRFKGSGSGTEFTLTISDLECADAATYYCLGYKSDDYTFGGGTKVEIK

SEQ ID NO: 78 - protein, 118 aa, synthetic construct
  REGION 1..118: note = Synthetic polypeptide
QSLEESGGRLVTPGGSLTLTCTVSGIDLSSYAMSWVRQAPEKGLEWIGFINNYGTYYASWAKGRFTISKTSTTVDLKVTSLTTEDTATYFCVRGGRSPNYDIVSGDIWGPGTLVTVSS

SEQ ID NO: 79 - protein, 110 aa, synthetic construct; identical to SEQ ID NO: 7
  REGION 1..110: note = Synthetic polypeptide

SEQ ID NO: 80 - protein, 118 aa, synthetic construct; identical to SEQ ID NO: 78
  REGION 1..118: note = Synthetic polypeptide

SEQ ID NO: 81 - protein, 110 aa, synthetic construct; identical to SEQ ID NO: 7
  REGION 1..110: note = Synthetic polypeptide

SEQ ID NO: 82 - protein, 119 aa, synthetic construct; identical to SEQ ID NO: 6
  REGION 1..119: note = Synthetic polypeptide

SEQ ID NO: 83 - protein, 110 aa, synthetic construct; identical to SEQ ID NO: 7
  REGION 1..110: note = Synthetic polypeptide

SEQ ID NO: 84 - protein, 115 aa, synthetic construct; identical to SEQ ID NO: 76
  REGION 1..115: note = Synthetic polypeptide

SEQ ID NO: 85 - protein, 109 aa, synthetic construct; identical to SEQ ID NO: 77
  REGION 1..109: note = Synthetic polypeptide

SEQ ID NO: 86 - protein, 115 aa, synthetic construct; identical to SEQ ID NO: 10
  REGION 1..115: note = Synthetic polypeptide

SEQ ID NO: 87 - protein, 109 aa, synthetic construct; identical to SEQ ID NO: 77
  REGION 1..109: note = Synthetic polypeptide

SEQ ID NO: 88 - protein, 115 aa, synthetic construct; identical to SEQ ID NO: 10
  REGION 1..115: note = Synthetic polypeptide

SEQ ID NO: 89 - protein, 109 aa, synthetic construct; identical to SEQ ID NO: 77
  REGION 1..109: note = Synthetic polypeptide

SEQ ID NO: 90 - protein, 118 aa, synthetic construct
  REGION 1..118: note = Synthetic polypeptide
QSLEESGGRLVTPGTPLTLTCTVSGFSLNNYYMNWVRQAPGKGLEWIGIIYPDIDTTDYASWVKGRFTISKTSTTVDLKITSPTTEDTATYFCARSDIDYYTTRLDLWGQGTLVTISS

SEQ ID NO: 91 - protein, 111 aa, synthetic construct
  REGION 1..111: note = Synthetic polypeptide
AQVLTQTPSPVSAAVGGTVSINCQSSPSVYNNNWLSWFQQKPGQPPKLLIYGASTLASGVPSRFKGSGSGTQFTLTISDVQCDDAATYYCAGGYDSNSDTAFGGGTELEIL

SEQ ID NO: 92 - protein, 5 aa, synthetic construct
  REGION 1..5: note = Synthetic polypeptide
SYHMS

SEQ ID NO: 93 - protein, 16 aa, synthetic construct
  REGION 1..16: note = Synthetic polypeptide
IIYRSGNTYSANWAKG

SEQ ID NO: 94 - protein, 10 aa, synthetic construct
  REGION 1..10: note = Synthetic polypeptide
ESSTFYGMDL

SEQ ID NO: 95 - protein, 13 aa, synthetic construct
  REGION 1..13: note = Synthetic polypeptide
QASQSVYGNNELA

SEQ ID NO: 96 - protein, 7 aa, synthetic construct
  REGION 1..7: note = Synthetic polypeptide
RASTLAS

SEQ ID NO: 97 - protein, 9 aa, synthetic construct
  REGION 1..9: note = Synthetic polypeptide
LGYKSDDYT

SEQ ID NO: 98 - protein, 5 aa, synthetic construct
  REGION 1..5: note = Synthetic polypeptide
SYAMS

SEQ ID NO: 99 - protein, 15 aa, synthetic construct
  REGION 1..15: note = Synthetic polypeptide
FINNYGTYYASWAKG

SEQ ID NO: 100 - protein, 14 aa, synthetic construct
  REGION 1..14: note = Synthetic polypeptide
GGRSPNYDIVSGDI

SEQ ID NO: 101 - protein, 11 aa, synthetic construct
  REGION 1..11: note = Synthetic polypeptide
QASQNIYNSLA

SEQ ID NO: 102 - protein, 7 aa, synthetic construct
  REGION 1..7: note = Synthetic polypeptide
DASELAS

SEQ ID NO: 103 - protein, 12 aa, synthetic construct
  REGION 1..12: note = Synthetic polypeptide
QSSSAGDSYVGG

SEQ ID NO: 104 - protein, 15 aa, synthetic construct
  REGION 1..15: note = Synthetic polypeptide
FINMYGTYYASWAKG

SEQ ID NO: 105 - protein, 14 aa, synthetic construct
  REGION 1..14: note = Synthetic polypeptide
GGRSPDYDIVSGDI

SEQ ID NO: 106 - protein, 16 aa, synthetic construct
  REGION 1..16: note = Synthetic polypeptide
IIYRSGNTYYANWAKG

SEQ ID NO: 107 - protein, 5 aa, synthetic construct
  REGION 1..5: note = Synthetic polypeptide
NYYMN

SEQ ID NO: 108 - protein, 17 aa, synthetic construct
  REGION 1..17: note = Synthetic polypeptide
IIYPDIDTTDYASWVKG

SEQ ID NO: 109 - protein, 12 aa, synthetic construct
  REGION 1..12: note = Synthetic polypeptide
SDIDYYTTRLDL

SEQ ID NO: 110 - protein, 12 aa, synthetic construct
  REGION 1..12: note = Synthetic polypeptide
SSPSVYNNNWLS

SEQ ID NO: 111 - protein, 7 aa, synthetic construct
  REGION 1..7: note = Synthetic polypeptide
GASTLAS

SEQ ID NO: 112 - protein, 11 aa, synthetic construct
  REGION 1..11: note = Synthetic polypeptide
AGGYDSNSDTA

SEQ ID NO: 113 - protein, 986 aa, Macaca mulatta
MAGIFYFALFSCLFGICDAVTGSRVYPANEVTLLDSRSVQGELGWIASPLEGGWEEVSIMDEKNTPIRTYQVCNVMEPSQNNWLRTDWITREGAQRVYIEIKFTLRDCNSLPGVMGTCKETFNLYYYESDNDKERFIRENQFVKIDTIAADESFTQVDIGDRIMKLNTEIRDVGPLSKKGFYLAFQDVGACIALVSVRVFYKKCPLTVRNLAQFPDTITGADTSSLVEVRGSCVNNSEEKDVPKMYCGADGEWLVPIGNCLCNAGHEERSGECQACKIGYYKALSTDATCAKCPPHSYSVWEGATSCTCDRGFFRADNDAASMPCTRPPSAPLNLISNVNETSVNLEWSSPQNTGGRQDISYNVVCKKCGAGDPSKCRPCGSGVHYTPQQNGLKTTKVSITDLLAHTNYTFEIWAVNGVSKYNPSPDQSVSVTVTTNQAAPSSIALVQAKEVTRYSVALAWLEPDRPNGVILEYEVKYYEKDQNERSYRIVRTAARNTDIKGLNPLTSYVFHVRARTAAGYGDFSEPLEVTTNTVPSRIIGDGANSTVLLVSVSGSVVLVVILIAAFVISRRRSKYSKAKQEADEEKHLNQGVRTYVDPFTYEDPNQAVREFAKEIDASCIKIEKVIGVGEFGEVCSGRLKVPGKREICVAIKTLKAGYTDKQRRDFLSEASIMGQFDHPNIIHLEGVVTKCKPVMIITEYMENGSLDAFLRKNDGRFTVIQLVGMLRGIGSGMKYLSDMSYVHRDLAARNILVNSNLVCKVSDFGMSRVLEDDPEAAYTTRGGKIPIRWTAPEAIAYRKFTSASDVWSYGIVMWEVMSYGERPYWDMSNQDVIKAIEEGYRLPPPMDCPIALHQLMLDCWQKERSDRPKFGQIVNMLDKLIRNPNSLKRTGTESSRPNTALLDPSSPEFSAVVSVGDWLQAIKMDRYKDNFTAAGYTTLEAVVHVNQEDLARIGITAITHQNKILSSVQAMRTQMQQMHGRMVPV

SEQ ID NO: 114 - protein, 528 aa, Macaca mulatta
VTGSRVYPANEVTLLDSRSVQGELGWIASPLEGGWEEVSIMDEKNTPIRTYQVCNVMEPSQNNWLRTDWITREGAQRVYIEIKFTLRDCNSLPGVMGTCKETFNLYYYESDNDKERFIRENQFVKIDTIAADESFTQVDIGDRIMKLNTEIRDVGPLSKKGFYLAFQDVGACIALVSVRVFYKKCPLTVRNLAQFPDTITGADTSSLVEVRGSCVNNSEEKDVPKMYCGADGEWLVPIGNCLCNAGHEERSGECQACKIGYYKALSTDATCAKCPPHSYSVWEGATSCTCDRGFFRADNDAASMPCTRPPSAPLNLISNVNETSVNLEWSSPQNTGGRQDISYNVVCKKCGAGDPSKCRPCGSGVHYTPQQNGLKTTKVSITDLLAHTNYTFEIWAVNGVSKYNPSPDQSVSVTVTTNQAAPSSIALVQAKEVTRYSVALAWLEPDRPNGVILEYEVKYYEKDQNERSYRIVRTAARNTDIKGLNPLTSYVFHVRARTAAGYGDFSEPLEVTTNTVPSRIIGDGANST

SEQ ID NO: 115 - protein, 986 aa, Oryctolagus cuniculus
MAGIFYFVFFSFLFGVCDAVTGSRVYPANEVTLLDSRSVQGELGWIASPLEGGWEEVSIMDEKNTPIRTYQVCNVMEPSQNNWLRTDWITREGAQRVYIEIKFTLRDCNSLPGVMGTCKETFNLYYYESDNDKERFIRESQFAKIDTIAADESFTQVDIGDRIMKLNTEIRDVGPLSRKGFYLAFQDVGACIALVSVRVFYKKCPLTVRNLAQFPDTITGADTSSLVEVRGSCVNNSEEKDVPKMYCGADGEWLVPIGNCLCNAGHEEQSGECQACKIGYYKALSTDATCAKCPPHSYSVWEGATSCTCDRGFFRADNDAASMPCTRPPSAPLNLISNVNETSVNLEWSSPQNTGGRQDISYNVVCKKCGAGDPSKCRPCGSGVHYTPQQNGLKSTKVSITDLLAHTNYTFEIWAVNGVSKYNPSPDQSVSVTVTTNQAAPSSIALVQAKEVTRYSVALAWLEPDRPNGVILEYEVKYYEKDQNERSYRIVRTAARNTDIKGLNPLTSYVFHVRARTAAGYGDFSEPLEVTTNTVPSRIIGDGANSTVLLVSVSGSVVLVVILIAAFVISRRRSKYSKAKQEADEEKHLNQGVRTYVDPFTYEDPNQAVREFAKEIDASCIKIEKVIGVGEFGEVCSGRLKVPGKREICVAIKTLKAGYTDKQRRDFLSEASIMGQFDHPNIIHLEGVVTKCKPVMIITEYMENGSLDAFLRKNDGRFTVIQLVGMLRGIGSGMKYLSDMSYVHRDLAARNILVNSNLVCKVSDFGMSRVLEDDPEAAYTTRGGKIPIRWTAPEAIAYRKFTSASDVWSYGIVMWEVMSYGERPYWDMSNQDVIKAIEEGYRLPPPMDCPIALHQLMLDCWQKERSDRPKFGQIVNMLDKLIRNPNSLKRTGTESSRPNTALLDPSSPEFSAVVSVGDWLQAIKMDRYKDNFTAAGYTTLEAVVHMNQDDLSRIGITAITHQNKILSSVQAMRTQMQQMHGRMVPV

SEQ ID NO: 116 - protein, 528 aa, Oryctolagus cuniculus
VTGSRVYPANEVTLLDSRSVQGELGWIASPLEGGWEEVSIMDEKNTPIRTYQVCNVMEPSQNNWLRTDWITREGAQRVYIEIKFTLRDCNSLPGVMGTCKETFNLYYYESDNDKERFIRESQFAKIDTIAADESFTQVDIGDRIMKLNTEIRDVGPLSRKGFYLAFQDVGACIALVSVRVFYKKCPLTVRNLAQFPDTITGADTSSLVEVRGSCVNNSEEKDVPKMYCGADGEWLVPIGNCLCNAGHEEQSGECQACKIGYYKALSTDATCAKCPPHSYSVWEGATSCTCDRGFFRADNDAASMPCTRPPSAPLNLISNVNETSVNLEWSSPQNTGGRQDISYNVVCKKCGAGDPSKCRPCGSGVHYTPQQNGLKSTKVSITDLLAHTNYTFEIWAVNGVSKYNPSPDQSVSVTVTTNQAAPSSIALVQAKEVTRYSVALAWLEPDRPNGVILEYEVKYYEKDQNERSYRIVRTAARNTDIKGLNPLTSYVFHVRARTAAGYGDFSEPLEVTTNTVPSRIIGDGANST

SEQ ID NO: 117 - protein, 986 aa, Rattus norvegicus
MAGIFYFILFSFLFGICDAVTGSRVYPANEVTLLDSRSVQGELGWIASPLEGGWEEVSIMDEKNTPIRTYQVCNVMEASQNNWLRTDWITREGAQRVYIEIKFTLRDCNSLPGVMGTCKETFNLYYYESDNDKERFIRESQFGKIDTIAADESFTQVDIGDRIMKLNTEIRDVGPLSKKGFYLAFQDVGACIALVSVRVFYKKCPLTVRNLAQFPDTITGADTSSLVEVRGSCVNNSEEKDVPKMYCGADGEWLVPIGNCLCNAGHEEQNGECQACKIGYYKALSTDATCAKCPPHSYSVWEGATSCTCDRGFFRADNDAASMPCTRPPSAPLNLISNVNETSVNLEWSSPQNTGGRQDISYNVVCKKCGAGDPSKCRPCGSGVHYTPQQNGLKTTRVSITDLLAHTNYTFEIWAVNGVSKYNPSPDQSVSVTVTTNQAAPSSIALVQAKEVTRYSVALAWLEPDRPNGVILEYEVKYYEKDQNERSYRIVRTAARNTDIKGLNPLTSYVFHVRARTAAGYGDFSEPLEVTTNTVPSRIIGDGANSTVLLVSVSGSVVLVVILIAAFVISRRRSKYSQAKQEADEEKHLNQGVRTYVDPFTYEDPNQAVREFAKEIDASCIKIEKVIGVGEFGEVCSGRLKVPGKREICVAIKTLKAGYTDKQRRDFLSEASIMGQFDHPNIIHLEGVVTKCKPVMIITEYMENGSLDAFLRKNDGRFTVIQLVGMLRGIGSGMKYLSDMSYVHRDLAARNILVNSNLVCKVSDFGMSRVLEDDPEAAYTTRGGKIPIRWTAPEAIAYRKFTSASDVWSYGIVMWEVMSYGERPYWDMSNQDVIKAIEEGYRLPPPMDCPIALHQLMLDCWQKERSDRPKFGQIVNMLDKLIRNPNSLKRTGPESSRPNTALLDPSSPEFSAVVSVGDWLQAIKMDRYKDNFTAAGYTTLEAVVHMSQDDLARIGITAITHQNKILSSVQAMRTQMQQMHGRMVPV

SEQ ID NO: 118 - protein, 528 aa, Rattus norvegicus
VTGSRVYPANEVTLLDSRSVQGELGWIASPLEGGWEEVSIMDEKNTPIRTYQVCNVMEASQNNWLRTDWITREGAQRVYIEIKFTLRDCNSLPGVMGTCKETFNLYYYESDNDKERFIRESQFGKIDTIAADESFTQVDIGDRIMKLNTEIRDVGPLSKKGFYLAFQDVGACIALVSVRVFYKKCPLTVRNLAQFPDTITGADTSSLVEVRGSCVNNSEEKDVPKMYCGADGEWLVPIGNCLCNAGHEEQNGECQACKIGYYKALSTDATCAKCPPHSYSVWEGATSCTCDRGFFRADNDAASMPCTRPPSAPLNLISNVNETSVNLEWSSPQNTGGRQDISYNVVCKKCGAGDPSKCRPCGSGVHYTPQQNGLKTTRVSITDLLAHTNYTFEIWAVNGVSKYNPSPDQSVSVTVTTNQAAPSSIALVQAKEVTRYSVALAWLEPDRPNGVILEYEVKYYEKDQNERSYRIVRTAARNTDIKGLNPLTSYVFHVRARTAAGYGDFSEPLEVTTNTVPSRIIGDGANST

SEQ ID NO: 119 - protein, 986 aa, Mus musculus
MAGIFYFILFSFLFGICDAVTGSRVYPANEVTLLDSRSVQGELGWIASPLEGGWEEVSIMDEKNTPIRTYQVCNVMEASQNNWLRTDWITREGAQRVYIEIKFTLRDCNSLPGVMGTCKETFNLYYYESDNDKERFIRESQFGKIDTIAADESFTQVDIGDRIMKLNTEIRDVGPLSKKGFYLAFQDVGACIALVSVRVFYKKCPLTVRNLAQFPDTITGADTSSLVEVRGSCVNNSEEKDVPKMYCGADGEWLVPIGNCLCNAGHEEQNGECQACKIGYYKALSTDASCAKCPPHSYSVWEGATSCTCDRGFFRADNDAASMPCTRPPSAPLNLISNVNETSVNLEWSSPQNTGGRQDISYNVVCKKCGAGDPSKCRPCGSGVHYTPQQNGLKTTRVSITDLLAHTNYTFEIWAVNGVSKYNPSPDQSVSVTVTTNQAAPSSIALVQAKEVTRYSVALAWLEPDRPNGVILEYEVKYYEKDQNERSYRIVRTAARNTDIKGLNPLTSYVFHVRARTAAGYGDFSEPLEVTTNTVPSRIIGDGANSTVLLVSVSGSVVLVVILIAAFVISRRRSKYSKAKQEADEEKHLNQGVRTYVDPFTYEDPNQAVREFAKEIDASCIKIEKVIGVGEFGEVCSGRLKVPGKREICVAIKTLKAGYTDKQRRDFLSEASIMGQFDHPNIIHLEGVVTKCKPVMIITEYMENGSLDAFLRKNDGRFTVIQLVGMLRGIGSGMKYLSDMSYVHRDLAARNILVNSNLVCKVSDFGMSRVLEDDPEAAYTTRGGKIPIRWTAPEAIAYRKFTSASDVWSYGIVMWEVMSYGERPYWDMSNQDVIKAIEEGYRLPPPMDCPIALHQLMLDCWQKERSDRPKFGQIVNMLDKLIRNPNSLKRTGSESSRPNTALLDPSSPEFSAVVSVGDWLQAIKMDRYKDNFTAAGYTTLEAVVHMSQDDLARIGITAITHQNKILSSVQAMRTQMQQMHGRMVPV

SEQ ID NO: 120 - protein, 528 aa, Mus musculus
VTGSRVYPANEVTLLDSRSVQGELGWIASPLEGGWEEVSIMDEKNTPIRTYQVCNVMEASQNNWLRTDWITREGAQRVYIEIKFTLRDCNSLPGVMGTCKETFNLYYYESDNDKERFIRESQFGKIDTIAADESFTQVDIGDRIMKLNTEIRDVGPLSKKGFYLAFQDVGACIALVSVRVFYKKCPLTVRNLAQFPDTITGADTSSLVEVRGSCVNNSEEKDVPKMYCGADGEWLVPIGNCLCNAGHEEQNGECQACKIGYYKALSTDASCAKCPPHSYSVWEGATSCTCDRGFFRADNDAASMPCTRPPSAPLNLISNVNETSVNLEWSSPQNTGGRQDISYNVVCKKCGAGDPSKCRPCGSGVHYTPQQNGLKTTRVSITDLLAHTNYTFEIWAVNGVSKYNPSPDQSVSVTVTTNQAAPSSIALVQAKEVTRYSVALAWLEPDRPNGVILEYEVKYYEKDQNERSYRIVRTAARNTDIKGLNPLTSYVFHVRARTAAGYGDFSEPLEVTTNTVPSRIIGDGANST

SEQ ID NO: 121 - protein, 19 aa, Homo sapiens
MAGIFYFALFSCLFGICDA

SEQ ID NO: 122 - protein, 15 aa, Homo sapiens
MSALLILALVGAAVA

SEQ ID NO: 123 - protein, 190 aa, Homo sapiens
VTGSRVYPANEVTLLDSRSVQGELGWIASPLEGGWEEVSIMDEKNTPIRTYQVCNVMEPSQNNWLRTDWITREGAQRVYIEIKFTLRDCNSLPGVMGTCKETFNLYYYESDNDKERFIRENQFVKIDTIAADESFTQVDIGDRIMKLNTEIRDVGPLSKKGFYLAFQDVGACIALVSVRVFYKKCPLTVR

SEQ ID NO: 124 - protein, 114 aa, Homo sapiens
TRPPSAPLNLISNVNETSVNLEWSSPQNTGGRQDISYNVVCKKCGAGDPSKCRPCGSGVHYTPQQNGLKTTKVSITDLLAHTNYTFEIWAVNGVSKYNPNPDQSVSVTVTTNQA

SEQ ID NO: 125 - protein, 112 aa, Homo sapiens
TNQAAPSSIALVQAKEVTRYSVALAWLEPDRPNGVILEYEVKYYEKDQNERSYRIVRTAARNTDIKGLNPLTSYVFHVRARTAAGYGDFSEPLEVTTNTVPSRIIGDGANST

SEQ ID NO: 126 - protein, 374 aa, synthetic construct
  REGION 1..374: note = Synthetic polypeptide
EEGKLVIWINGDKGYNGLAEVGKKFEKDTGIKVTVEHPDKLEEKFPQVAATGDGPDIIFWAHDRFGGYAQSGLLAEITPDKAFQDKLYPFTWDAVRYNGKLIAYPIAVEALSLIYNKDLLPNPPKTWEEIPALDKELKAKGKSALMFNLQEPYFTWPLIAADGGYAFKYENGKYDIKDVGVDNAGAKAGLTFLVDLIKNKHMNADTDYSIAEAAFNKGETAMTINGPWAWSNIDTSKVNYGVTVLPTFKGQPSKPFVGVLSAGINAASPNKELAKEFLENYLLTDEGLEAVNKDKPLGAVALKSYEEELAKDPRIAATMENAQKGEIMPNIPQMSAFWYAVRTAVINAASGRQTVDEALKDAQTHHHHHHHHHH